European Patent Specification EP 3 609 331 B1, published December 18, 2024. Title: A SYNERGISTIC COMPOSITION OF A NEMATICIDE. Applicant: TELLURIS BIOTECH INDIA PRIVATE LIMITED. The sequence listing filed with the application follows.

SEQUENCE LISTING (4 sequences)

SEQ ID NO: 1 - protein, 549 aa, Caenorhabditis elegans
MLCEIECRALSTAHTRLIHDFEPRDALTYLEGKNIFTEDHSELISKMSTRLERIANFLRIYRRQASELGPLIDFFNYNNQSHLADFLEDYIDFAINEPDLLRPVVIAPQFSRQMLDRKLLLGNVPKQMTCYIREYHVDRVIKKLDEMCDLDSFFLFLHGRAGSGKSVIASQALSKSDQLIGINYDSIVWLKDSGTAPKSTFDLFTDILLMLKSEDDLLNFPSVEHVTSVVLKRMICNALIDRPNTLFVFDDVVQEETIRWAQELRLRCLVTTRDVEISNAASQTCEFIEVTSLEIDECYDFLEAYGMPMPVGEKEEDVLNKTIELSSGNPATLMMFFKSCEPKTFEKMAQLNNKLESRGLVGVECITPYSYKSLAMALQRCVEVLSDEDRSALAFAVVMPPGVDIPVKLWSCVIPVDICSNEEEQLDDEVADRLKRLSKRGALLSGKRMPVLTFKIDHIIHMFLKHVVDAQTIANGISILEQRLLEIGNNNVSVPERHIPSHFQKFRRSSASEMYPKTTEETVIRPEDFPKFMQLHQKFYDSLKNFACC

SEQ ID NO: 2 - protein, 15 aa, Caenorhabditis elegans
DLLRPVVIAPQFSRQ

SEQ ID NO: 3 - protein, 19 aa, Caenorhabditis elegans
RQMLDRKLLLGNVPKQMTC

SEQ ID NO: 4 - protein, 12 aa, Caenorhabditis elegans
FPKFMQLHQKFY